European Patent Application EP 4 631 570 A2, published October 15, 2025. Title: MicroRNA-targeted therapy for cardiac repair. Applicant: Charite-Universitätsmedizin Berlin. Application EP. The sequence listing filed with the application follows.

SEQUENCE LISTING (6 sequences)

SEQ ID NO: 1 - protein, 22 aa, Homo sapiens
GAGUGCCUUCUUUUGGAGCGUU

SEQ ID NO: 2 - protein, 21 aa, Homo sapiens
AAGUGCCUCCUUUUAGAGUGU

SEQ ID NO: 3 - protein, 22 aa, Homo sapiens
AUCGUGCAUCCUUUUAGAGUGU

SEQ ID NO: 4 - protein, 22 aa, Homo sapiens
AUCGUGCAUCCCUUUAGAGUGU

SEQ ID NO: 5 - protein, 23 aa, Homo sapiens
AAGUGCCGCCAUCUUUUGAGUGU

SEQ ID NO: 6 - protein, 20 aa, Homo sapiens
UGAGGAGAUGCUGGGACUGA